European Patent Application EP 4 353 748 A1, published April 17, 2024. Title: 新型抗栓抗体. Applicant: 上海循曜生物科技有限公司. The sequence listing filed with the application follows.

SEQUENCE LISTING (20 sequences)

SEQ ID NO: 1 - protein, 120 aa, (Mus musculus)
QVTLKESGPGILKPSQTLSLTCSFSGFSLNTPGMGVGWIRQPSGKGLEWLAHIWWDDDKYYNPSLKSQLTISKDTSRNQVFLKITSVDTADTATYYCARSDDVSYALDYWGQGTSVTVSS

SEQ ID NO: 2 - protein, 107 aa, (Mus musculus)
DIQMTQSPASLSASVGETVTITCRASENIDSYLAWYQQKQGKSPQLLVYNAKTLADGVPSRFSGSGSGTQFSLKIDSLQPEDFGSHYCQHHDGTTWTFGGGTKLEIK

SEQ ID NO: 3 - protein, 10 aa, (Mus musculus)
GFSLNTPGMG

SEQ ID NO: 4 - protein, 7 aa, (Mus musculus)
IWWDDDK

SEQ ID NO: 5 - protein, 12 aa, (Mus musculus)
ARSDDVSYALDY

SEQ ID NO: 6 - protein, 6 aa, (Mus musculus)
ENIDSY

SEQ ID NO: 7 - protein, 3 aa, (Mus musculus)
NAK

SEQ ID NO: 8 - protein, 9 aa, (Mus musculus)
QHHDGTTWT

SEQ ID NO: 9 - protein, 25 aa, (Mus musculus)
QVTLKESGPGILKPSQTLSLTCSFS

SEQ ID NO: 10 - protein, 17 aa, (Mus musculus)
VGWIRQPSGKGLEWLAH

SEQ ID NO: 11 - protein, 38 aa, (Mus musculus)
YYNPSLKSQLTISKDTSRNQVFLKITSVDTADTATYYC

SEQ ID NO: 12 - protein, 14 aa, (Mus musculus)
CARSDDVSYALDYW

SEQ ID NO: 13 - protein, 16 aa, (Mus musculus)
YALDYWGQGTSVTVSS

SEQ ID NO: 14 - protein, 11 aa, (Mus musculus)
WGQGTSVTVSS

SEQ ID NO: 15 - protein, 26 aa, (Mus musculus)
DIQMTQSPASLSASVGETVTITCRAS

SEQ ID NO: 16 - protein, 17 aa, (Mus musculus)
LAWYQQKQGKSPQLLVY

SEQ ID NO: 17 - protein, 36 aa, (Mus musculus)
TLADGVPSRFSGSGSGTQFSLKIDSLQPEDFGSHYC

SEQ ID NO: 18 - protein, 11 aa, (Mus musculus)
CQHHDGTTWTF

SEQ ID NO: 19 - protein, 12 aa, (Mus musculus)
WTFGGGTKLEIK

SEQ ID NO: 20 - protein, 10 aa, (Mus musculus)
FGGGTKLEIK